European Patent Application EP 4 302 780 A1, published January 10, 2024. Title: Composition for preventing or treating cerebrovascular disease. Applicant: Tokyo Metropolitan Institute of Medical Science The University of Tokyo. The sequence listing filed with the application follows.

SEQUENCE LISTING (5 sequences)

SEQ ID NO: 1 - DNA, 20 bp, Artificial Sequence
  Pla2g2e primer (F)
gaccccaagctggaaaagta

SEQ ID NO: 2 - DNA, 20 bp, Artificial Sequence
  Pla2g2e primer (R)
tagtgggcatacttgcggtt

SEQ ID NO: 3 - DNA, 20 bp, Artificial Sequence
  Gapdh primer (F)
aactttggcattgtggaagg

SEQ ID NO: 4 - DNA, 20 bp, Artificial Sequence
  Gapdh primer (R)
ggatgcagggatgatgttct

SEQ ID NO: 5 - DNA, 6466 bp, Mus musculus
aatccatcagcagcggtcgtattagccaaacacttgaactcccgctgcctgcaggatgcatagctgtattgcttcatatgcgcggggtgaaaggtcatacagactgtgggccatctgtaccccacacggttgattacatggatgaaccccgctaacagcacggcattgggaaactagtcacggaggcatagggtatccatccatcaacacaaaggcaagcgcaaacaatactgtaaaacccataaagaaaaacaaggacataagagctggaaaggctgacacggttgtggctggggtggaggggcacagtcagggacgacatgaccacagacgtctcctaaaggccggttctttagctgcatgacgtcagcgcagacttcagctcagcagtctttaaagttcccataggtttgcacatcctcctgacgattggtatgttgtaggattttaagagacggtggctgataaggagaatgtggaatgcgcacgtgagcagatcaagctgagctcgtggcaggcattgggcaactgggcagcgcacagagaaggagttctgggatgctgctggcaaggggccagctgcctggagcttccgagagcaagataacatcgcaccgtcaatcacgccgccatgccaaggccagaagaggccctgagtgagcgggtggaggacagctgtgtcaatagtttcacatatcctggtgacagctagtggactaaaaagggagaggaggtggttgggtcacactggaagtctagtcagggttcttcctcccaactccccagctgggtgccagagtccgtgagcccattagcatatgtacagagtttctctctctctctctctctctctctctctctctctctctctcccctctctctctccctctccctccccctctccctctctctctccctctctccctccttccctccacctgtcaggctgtctgtggttgtgtgttctgtctgtctctctgactgtggttgtgtgttctctctgtgtctgtctgtctgtctgtctgtctgtctgtctatctgtgattgtgtgtgtctatttatggttgtgtgctcccagctctcctcttcctcctcttcttcctcttcctcctcttcctcctccttggcgactggagagatggctctgtgactaagagcacttgctgctctcacagaggacccaggttcagttcccagcaccaggcagctcacagccacctgtaactctagttccaggggatccaacgccctctgcatggtcctgggttctataagaaagcaggcagagcaagccatgcagaacaagccagtgagcagcatccttccatagtgtgtgtgtgtgtgtgttaccgtttctgctgccaagatgaaacactgtaaccaaagagcaagttgcgaaggaaagggcttgttagacttacacttccgtaacactcactgtgcatcactgaaagagtcaggacaggaactcagtcaagcagggcaggaacctggaggcaggagctcatgagaggccatggaaggatgctgctcactggcttgttctgcatggcttgctctgcctgctttcttatagaacccaggaccatcagcccagggatggccccgcccacaatagtctgggccttcccaccattcactaagtctgaaaattccctacaggtgaatctcaggaatttctcaatggaggttctctcctttcagatgacgctatattgtgtcagtttgacacaaggctagccagcatagcgtgtagtgtgccttcatgagttcatacacagcacaagtgttgcaggtgcctgtggggagcattgagtaccagtttctctggagttacagatctgggagcaaacttatttcgtaccctctttagtgcccgtgatggccactcctcacctaccagcacctgacgtgacccgctgtgactgtcactgaggtctttggggatgtgatgtaagaaaccactagctttcagcacctcagcgctcagagtgtcatcagacagtctctgaggcctggggcagagcttccctgggctcctgtaaccgtctacctgacgttcccaccagtgcatctgaaaaatgccttcatttatgagtgtgttttgttttgtttctatgtagccctggctggtctagaacttgatatatagaccaggctggcttcaaactcacagagatccgcctgcctctgcctccacagtactggaatccaaggcgtgcaccagcaccaccacccagcccagaacaacctcttatttctggcctttgtgttacatctccactgtcagatctgagcgtcaggggtggaacaagcgctggattctcattgtgtgatcttacagactctttctctctaggagtgagacagtcacccggagctcagggtacagccagtagccctggaatattctctgtactcaggggccatattagccagccatcaaaatgtaactggcctgccagagaaaaggatattttagagactcttgcgtctctccatttgactatcagactagtgaaatggtgggccactccaacactggaatccccctgggtaccttgtggtaggcaaaggaaaaggctgggaactcgtctcccagaaaagacttcccactgtgccaacaacttactagactccccttctgaagaaattggagcccagataatgacaggtcagcggtcggcggggatcatggcatgcttagatgtgcagatccctgcccctccagttaaaagttaatgaacttttaaattttattttaatttatgtgtctgtgtgtctctctgtgtgtggctcacagtggccagaagagggcgtcagatctcctgtaagtggagttacagagagttgtaaaccgccctgtgggtaccaggaatcgaactcaggtcctctgcaagagcagcaagccctcttattcgctgagccgctgtctctggcccgatgtttaaatttcagtctcacttcagaaccctgacaaaggacttgagaggctcactgtatttctttgaccctctttctagagtggccacattaactagatctccttttcctgttttttgtttgtttgtttgtttgtttgtttttgatagttatgtggttgcattaattggcttctcaaaatcgggtggctccacctggcttcttgggtcacatagactatgaccccaggtttggtaacaataacattctaaagaagccaaggtttgaatctttgagacctagaagataatgtatttgccagtggcaggaggaattgcacagacagacagacagacagacagacagacagacactgcgcctaggagagcaggagagcagccaaggagtgcaagcatggcttgcaccatggctacttctgtaactaccagcttgctcattctacaccacaggacccttgagccacaaacaacaatgagtgaccctgctttaacaatgggggagcttggtgatgtctgaaagacagggagcaaaagcactgaggagccaagaagccccaggccgtgctggccacacctggccattgtgccacccagccctgcccagcaaccttttgctgggtgggaatccattgggcaaacaaacaggctcaggaagagaatcacccacgcacgccagaggaaagtgtaggtgtctgtgttattctaaacccggcccaggttcaagttcagatgtcaatgttacttctgaaggctgccggctcagccctcaagttgtcattggagagatgcaaacgagggctttacagtcaaagcccaggggtgaatcttcaaagtagctcagcatctgcaaggcctgctgattaaggccggatacccaacatctgaagcatctgccggtcacatcagtgacatccgtggctgtgacacggtggaaacagaaaccaaacaaacagggatgggacagggatgacgaggagtgggctcaggtaggtgtggttcgataaagtcattcgaaaagcaagcgtctgactctgtgagcccacttccggaggggggggggcgtagaaagataaatcagtattccagagagcggccgtaagtcagatgctcatcagaaagggcaggctaaagaaaatgtgacagaaacacagtttcctactttcctacatgaagagatagcttgactgcagccatcatttaacaatgactaccttgggtcagcaagatggctcagtgggtaaaggagcttgccgccaaaactcatgacctgagtttgatccccagaacctatgtagaggtggcaggggagatcagatggacagacctgtcctctgcccttcatgcatgcctgcgtcacacaataacaataacaacaataataataaataatgatactacttctaataataatgatgatgataataataagttgttattattattatttaacaagaaaaacatcccacggcacactgtgcatcttaaaaacatacagttctcaactgcgtgggtaagtctggggtgacggctcagtcagtgaagtgcttgccttgcaagccggaggatctgcatttggctccccgacacccacttaaaaaggcaggtgcagtggcgggacctgtgagtcagagacaagcgatttgtagagtcagcaagtccagccaatcagggttcagtaagagaccctgtctcaaaacatcaaataactctcaacggaggaagatgttcaacactgtgccatggcttctctgtgctctcacgagggctcatgcacactcacacagatgtgcacatgtgtgtcacacatatgtaaggccctgcggggtggaggcccacacttgaatcccagcgctgaggaagcagaaacacattcttctgggactcactggaagccagcagagtggacttcgtgggttgcggccaatgagagatcctgtctcaaaactcaggggccgggcggtggtggcgcacacctttaatcccagcacttgggaggcagaggcaggcggatttctgagttcaaggccagcctggtctacagagtgagttctaggacagccagggctatacagagaaaccctgtcttgaaaaaaacaaaaaataaaaataaaaaaaaatcaggctggggaccagggagatgatatttgccagaaagcttggtgacctggggttcaatgcccaggactcacatggtggagggacaggagggacaaaacagactcctaccatgtctttatactatggctggtggcctggctcctgtaccaaaccccctgaggacagaaagggaccctggtcctaactcctatttagggatcacgggacccaggagcctttttttggcctctcagacccccagtagcctcctgtccagcacacacatgtgctgagctctggggacgctggccaggaggccatgggctcaggtctaccgaatcctgcggcctttgatgtggagccaaaggagaccctacagccccccaaacaccctgtgctctcggcagcctccgagacagacacaccctctctgggtgctccctgttaggacttgtcatccccacccccagttcaccccatgagcagacagccctggcaccaggtgcagagccctcatgagtgccctcagggcgggcgcggcccacacccgcaccatctggtcttctgggggaggtcctgtagaggcagatacccagggtatgcagcaaacctcacctctaggttgggtaacatggtttcccctcccagccgtgcccatggcccccactactttttcctctctgtgcttcagctttcccttctataaaatgggctggcagtcaactgccctcggatgcttggtgttacagtgagaagcctttgtcttaaggtttgaaaagaccacgtcaccaggacagactgctaataaaggccctaccctgtggccagcttctgttcaaatccttactggctgcagagcctcctctaccctgggcctcagtttcttcatctggaaagtgggtgtgatgatgtgagctgacctcagagatgcttcaaggatgaagtgggggaagggactgcaacagcttgagtttcacagactgtcctgggagcatttcagcggagagcaagtcccgaagagaagagtggggggtagggcggcgacctcagccacgcccagaatagccttctgtttagccttctcctgcctttctccccttctttccaatgtcttgttaagtgtgcttgggcaagatgtgcagtcctggcccaggcaggggtggctaagggcatagcctgtgctctcccctcacaggcttccgagtgccccactcttctgctgttgcaggcttcactgtggacacccatgggtgggtgggggggtcctgggtggcccagggtagaggaggctgtgcagccactggggcacctgagtggagaggggctgggcctccggggcagggcaggtgctgactcatgggctcgcctggcactataaaggaaccagcccaggggcttcctgctgcctgctgaccgagcgagcaagg